European Patent Application EP 4 768 575 A1, published July 1, 2026. Title: 니코틴아미드 뉴클레오티드 트랜스하이드로게나제의 변이체를 포함하는 미생물 및 이를 이용하여 Ｌ-아미노산을 생산하는 방법. Applicant: 씨제이제일제당 주식회사. The sequence listing filed with the application follows.

SEQUENCE LISTING (112 sequences)

SEQ ID NO: 1 - DNA, 35 bp, synthetic construct
  source 1..35: mol_type = other DNA
aattcgagctcggtacccaatggagctgaaagaat

SEQ ID NO: 2 - DNA, 30 bp, synthetic construct
  source 1..30: mol_type = other DNA
cttcctgatagtcccgggacattgtttttc

SEQ ID NO: 3 - DNA, 30 bp, synthetic construct
  source 1..30: mol_type = other DNA
gaaaaacaatgtcccgggactatcaggaag

SEQ ID NO: 4 - DNA, 38 bp, synthetic construct
  source 1..38: mol_type = other DNA
gtcgactctagaggatccccataaaaacaggcagagga

SEQ ID NO: 5 - DNA, 35 bp, synthetic construct
  source 1..35: mol_type = other DNA
cctgaaaaacaatgtcccaacgaccgagcctattg

SEQ ID NO: 6 - DNA, 20 bp, synthetic construct
  source 1..20: mol_type = other DNA
gttgtgtctcctctaaagat

SEQ ID NO: 7 - DNA, 39 bp, synthetic construct
  source 1..39: mol_type = other DNA
tctttagaggagacacaacatgcttattggtattccgag

SEQ ID NO: 8 - DNA, 41 bp, synthetic construct
  source 1..41: mol_type = other DNA
aaccaacttcctgatagtcccctacaggtgggagatgatct

SEQ ID NO: 9 - DNA, 472 bp, synthetic construct
  source 1..472: mol_type = other DNA
aacgaccgagcctattgggattaccattgaagccagtgtgagttgcatcacattggcttcaaatctgagactttaatttgtggattcacgggggtgtaatgtagttcataattaaccccattcgggggagcagatcgtagtgcgaacgatttcaggttcgttccctgcaaaaactatttagcgcaagtgttggaaatgcccccgtttggggtcaatgtccatttttgaatgtgtctgtatgattttgcatctgctgcgaaatctttgtttccccgctaaagttgaggacaggttgacacggagttgactcgacgaattatccaatgtgagtaggtttggtgcgtgagttggaaaaattcgccatactcgcccttgggttctgtcagctcaagaattcttgagtgaccgatgctctgattgacctaactgcttgacacattgcatttcctacaatctttagaggagacacaac

SEQ ID NO: 10 - protein, 513 aa, Corynebacterium variabile
MLIGIPREPQTLVAATPDTVGKLIKLGYDVAVQSGAGDQANHPDSQYESAGARIVGDDVWSTADIITTLDTPSAEQRAAMKPQATLIARLAPGRNDELVADLAAKNLTAMAMDTVPRISRAQAMDVLSSQANVAGYRAVIEAANTFGRLFTGQVTAAGKVPPATVYVIGTGVAGLAAIGTANSMGAVVKATDLRPETAEQVESMGAEFVAIPTASEKSDDGYAKEMTQDQAAAAAKLYAEQAARADIVITTANIPGRKSPVLLTAADVAAMTPGSVIVDMAAANGGNCELTVPGEVTETDNGVKIIGYTDLAGRLPAQSSQLYGQNIVNLFKLVTPGKDGRLVLDMDDEIVRGITVTQASATGSASDILWPPPPVKVSAAPAPAPAAATAAAEAEEEEPKGSGLWWKIVAGALGVALVLASPLSVTTNYMILMLAVVVGFYVITAVSHSLHTPLMSETNAISGIILVGAVLQVGSSNAAIAVLAFIAVVIASINIFGGFAVTRRMLAMFQGGN

SEQ ID NO: 11 - protein, 499 aa, Corynebacterium variabile
MNSFILATEVTNPDVSQDLLDWTDRISTLAYLVAALLFILALAGLSKQQSASRGNTFGIAGMTIALVATVFKAAVQSHADPENYNDAWVTILLVAVAMLIGAVIGIARASKVEMTGMPELIAMLHCFVGAAAVLIGVNSFIHAEHTSEAGYEKFHLGEVYLGIFIGAVTFTGSIIAYLKLSARMKGAPLTLPGRNLLNLAIIVLSVVGMVFFILTGTEEADNKAVAWTILGIMIVLALLLGLHLVAAIGGGDMPVVVSMLNSYSGWAAAAAGFMLANPLLIITGALVGSSGAYLSYIMCKAMNRSFISVILGGFGTEASSSDDRDYGTHTEITAEETAELLKGAKSVMITPGYGMAVAQAQYPVAAMVSKLREKGVDVTFGIHPVAGRLPGHMNVLLAEAKVPYDIVHEMDEVNDDFADIDVVLVIGANDTVNPIAEEPGSPLAGMPVLKVWEAKRVVVFKRSMGAGYAGVQNPLFFNENTDMLLGDAKDSVEKITSAL

SEQ ID NO: 12 - DNA, 1542 bp, Corynebacterium variabile
  source 1..1542: mol_type = other DNA
atgctgattggtattccccgtgaaccccagacccttgttgctgcgaccccggacaccgttggtaaactgattaaactcggctatgacgttgcagtgcagtccggcgccggtgatcaagctaaccacccagactcccagtacgaatctgctggcgcgcgcattgtgggtgatgacgtctggtccaccgcagacatcattaccaccctggacaccccttccgcagaacagcgtgcagccatgaagccacaagccaccttgatcgctcgccttgcgcctggccgtaacgatgagctggtggcagacctcgctgcgaaaaatctgaccgcaatggcaatggataccgttccgcgcatttcccgtgctcaggcgatggacgtgctctcctctcaagcaaacgttgcaggctaccgcgcagtgatcgaggcagcaaataccttcggccgtctgtttaccggtcaggtcaccgctgcgggtaaggttccacctgctaccgtctatgttattggcaccggtgtggcaggcttggcagccatcggcaccgcaaactctatgggcgcggtggtcaaagcaaccgatcttcgcccggaaaccgcagagcaggtggaatctatgggcgcagagttcgtcgctatccctaccgcgtccgaaaagtctgatgacggttacgccaaagagatgacccaggatcaagctgcggcagccgctaagctgtatgcagaacaggcggcacgcgccgacatcgtgattaccaccgcaaacattcctggccgtaaatccccggttctgctcaccgccgctgatgtggcggcaatgaccccaggttctgtgatcgtggatatggccgctgcgaacggcggtaattgcgaactgaccgttcctggcgaggtgaccgaaaccgataacggcgtgaagatcattggttacaccgacttggctggccgccttcctgcacagtcctctcaattgtatggtcagaacatcgtgaatctgttcaagctcgtcacccccggcaaagatggtcgcttggtccttgacatggatgacgaaattgtgcgtggcatcaccgtcacccaagcatccgccaccggttccgcttctgacatcctgtggccgcccccacctgttaaggtgtccgcagcccctgctcctgcaccagctgcggcaaccgccgctgcggaggcagaagaggaagagccaaagggctccggtctgtggtggaaaatcgtcgcaggcgccctcggtgtcgcactggttctcgcctcccctctctctgttaccaccaactacatgattttgatgcttgctgttgtggtcggcttttatgtcatcaccgcggttacccactccctgcacaccccactcatgtccgaaaccaatgctatttctggcatcattttggtgggtgcggtccttcaggttggctcctctaacgcagccatcgctgtcttggcgttcatcgcaattgttatcgcatccattaatatcttcggcggttttgctgtgacccgccgtatgcttgcgatgttccagggaggtaactga

SEQ ID NO: 13 - DNA, 1500 bp, Corynebacterium variabile
  source 1..1500: mol_type = other DNA
atgaactcttttattctggcgaccgaagtgaccaaccccgatgtgtctcaggatttgctggactggaccgaccgtatttctaccctcgcttaccttgtggcagccctgctcttcatcctcgctttggcgggtctgtctaagcagcaatccgctgcgcgcggcaacaccttcggtatcgctggtatgaccattgcgctcgttgcaaccgtgtttaaagcagccgtgcagtcccacgcagatccagagaactataatgacgcatgggtcaccatcttgcttgtcgcagttgccatgctgattggtgcagtcatcggcattgctcgcgcgtccaaggttgagatgaccggtatgccagaactcatcgccatgttgcactgcttcgtgggtgctgcggcagtgctgatcggcgtcaactcttttattcacgcggaacacacctccgaggcaggttacgaaaaattccaccttggcgaagtgtatctgggtatcttcattggcgcagtcacctttaccggctctatcattgcctaccttaagctgtccgcccgcatgaaaggtgctccgctcaccttgcccggccgtaacctgctcaatctcgcaatcattgtgttgtccgtggtcggtatggtcttctttatcctgaccggcaccgaagaggcagataacaaggcagttgcctggaccattcttggtatcatgattgtgctggccttgcttctgggtcttcacctggtcgcagctatcggtggtggtgacatgccggttgtggtctccatgctcaactcttactccggttgggcggcagccgctgcgggcttcatgttggctaatcccctcttgatcattaccggcgccctcgtcggttcctctggtgcttacttgtcctatatcatgtgtaaggctatgaaccgctctttcatctccgttattctgggtggctttggcaccgaagcgtcctcttccgatgaccgtgattatggcacccacaccgaggtcaccgcggaagagaccgcagaacttctgaagaacgccaaatccgttatgatcacccctggttacggtatggctgtggcacaggcacaatatcccgttgcagcaatggtgtccaagctgcgcgagaagggtgtggacgtcaccttcggcatccacccagtcgcaggtcgtctccctggccacatgaacgttctcttggccgaagctaaggtcccgtacgatattgttcacgaaatggacgaagtgaatgatgactttgccgacatcgacgttgtgctcgttattggcgccaacgataccgtgaatccaatcgctgaagagccaggttctcctattgcgggtatgccagtcttgaaggtttgggacgcaaaccgcgtcgttgtgttcaaacgctctatgggcgccggctacgctggcgttcaaaacccattgttctttaacgagaacaccgatatgcttctgggcgatgctaaggactctgtggaaaaaatcacctccgcgctgtaa

SEQ ID NO: 14 - DNA, 28 bp, synthetic construct
  source 1..28: mol_type = other DNA
gcaaatgctatttctggcatcattttgg

SEQ ID NO: 15 - DNA, 34 bp, synthetic construct
  source 1..34: mol_type = other DNA
ccagaaatagcatttgcttcggacatgagtgggg

SEQ ID NO: 16 - DNA, 24 bp, synthetic construct
  source 1..24: mol_type = other DNA
accaccttcggtatcgctggtatg

SEQ ID NO: 17 - DNA, 28 bp, synthetic construct
  source 1..28: mol_type = other DNA
cagcgataccgaaggtggtgccgcgcgc

SEQ ID NO: 18 - DNA, 25 bp, synthetic construct
  source 1..25: mol_type = other DNA
accctcgcaatcattgtgttgtccg

SEQ ID NO: 19 - DNA, 35 bp, synthetic construct
  source 1..35: mol_type = other DNA
acacaatgattgcgagggtgagcaggttacggccg

SEQ ID NO: 20 - DNA, 27 bp, synthetic construct
  source 1..27: mol_type = other DNA
gcatctggtgcttacttgtcctatatc

SEQ ID NO: 21 - DNA, 30 bp, synthetic construct
  source 1..30: mol_type = other DNA
aagtaagcaccagatgcaccgacgagggcg

SEQ ID NO: 22 - DNA, 26 bp, synthetic construct
  source 1..26: mol_type = other DNA
ttcatcatgtgtaaggctatgaaccg

SEQ ID NO: 23 - DNA, 38 bp, synthetic construct
  source 1..38: mol_type = other DNA
tagccttacacatgatgaaggacaagtaagcaccagag

SEQ ID NO: 24 - DNA, 25 bp, synthetic construct
  source 1..25: mol_type = other DNA
tgcgtgaatccaatcgctgaagagc

SEQ ID NO: 25 - DNA, 36 bp, synthetic construct
  source 1..36: mol_type = other DNA
agcgattggattcacgcaatcgttggcgccaataac

SEQ ID NO: 26 - DNA, 23 bp, synthetic construct
  source 1..23: mol_type = other DNA
tgcgctgaagagccaggttctcc

SEQ ID NO: 27 - DNA, 37 bp, synthetic construct
  source 1..37: mol_type = other DNA
cctggctcttcagcgcatggattcacggtatcgttgg

SEQ ID NO: 28 - DNA, 21 bp, synthetic construct
  source 1..21: mol_type = other DNA
tgcgcgggtatgccagtcttg

SEQ ID NO: 29 - DNA, 36 bp, synthetic construct
  source 1..36: mol_type = other DNA
gactggcatacccgcgcaaggagaacctggctcttc

SEQ ID NO: 30 - DNA, 25 bp, synthetic construct
  source 1..25: mol_type = other DNA
tgcccagtcttgaaggtttgggacg

SEQ ID NO: 31 - DNA, 38 bp, synthetic construct
  source 1..38: mol_type = other DNA
aaccttcaagactgggcaacccgcaataggagaacctg

SEQ ID NO: 32 - DNA, 22 bp, synthetic construct
  source 1..22: mol_type = other DNA
tgctacgctggcgttcaaaacc

SEQ ID NO: 33 - DNA, 33 bp, synthetic construct
  source 1..33: mol_type = other DNA
ttgaacgccagcgtagcaggcgcccatagagcg

SEQ ID NO: 34 - DNA, 20 bp, synthetic construct
  source 1..20: mol_type = other DNA
tgcgctggcgttcaaaaccc

SEQ ID NO: 35 - DNA, 33 bp, synthetic construct
  source 1..33: mol_type = other DNA
ggttttgaacgccagcgcagccggcgcccatag

SEQ ID NO: 36 - DNA, 26 bp, synthetic construct
  source 1..26: mol_type = other DNA
cctcgtcggtgcatctggtgcttact

SEQ ID NO: 37 - DNA, 27 bp, synthetic construct
  source 1..27: mol_type = other DNA
acaagtaagcaccagatgcaccgacga

SEQ ID NO: 38 - DNA, 26 bp, synthetic construct
  source 1..26: mol_type = other DNA
cctcgtcggttgctctggtgcttact

SEQ ID NO: 39 - DNA, 27 bp, synthetic construct
  source 1..27: mol_type = other DNA
acaagtaagcaccagagcaaccgacga

SEQ ID NO: 40 - DNA, 26 bp, synthetic construct
  source 1..26: mol_type = other DNA
cctcgtcggtgattctggtgcttact

SEQ ID NO: 41 - DNA, 27 bp, synthetic construct
  source 1..27: mol_type = other DNA
acaagtaagcaccagaatcaccgacga

SEQ ID NO: 42 - DNA, 26 bp, synthetic construct
  source 1..26: mol_type = other DNA
cctcgtcggtgaatctggtgcttact

SEQ ID NO: 43 - DNA, 27 bp, synthetic construct
  source 1..27: mol_type = other DNA
acaagtaagcaccagattcaccgacga

SEQ ID NO: 44 - DNA, 26 bp, synthetic construct
  source 1..26: mol_type = other DNA
cctcgtcggtttctctggtgcttact

SEQ ID NO: 45 - DNA, 27 bp, synthetic construct
  source 1..27: mol_type = other DNA
acaagtaagcaccagagaaaccgacga

SEQ ID NO: 46 - DNA, 26 bp, synthetic construct
  source 1..26: mol_type = other DNA
cctcgtcggtggctctggtgcttact

SEQ ID NO: 47 - DNA, 27 bp, synthetic construct
  source 1..27: mol_type = other DNA
acaagtaagcaccagagccaccgacga

SEQ ID NO: 48 - DNA, 26 bp, synthetic construct
  source 1..26: mol_type = other DNA
cctcgtcggtcactctggtgcttact

SEQ ID NO: 49 - DNA, 27 bp, synthetic construct
  source 1..27: mol_type = other DNA
acaagtaagcaccagagtgaccgacga

SEQ ID NO: 50 - DNA, 26 bp, synthetic construct
  source 1..26: mol_type = other DNA
cctcgtcggtatctctggtgcttact

SEQ ID NO: 51 - DNA, 27 bp, synthetic construct
  source 1..27: mol_type = other DNA
acaagtaagcaccagagataccgacga

SEQ ID NO: 52 - DNA, 26 bp, synthetic construct
  source 1..26: mol_type = other DNA
cctcgtcggtaagtctggtgcttact

SEQ ID NO: 53 - DNA, 27 bp, synthetic construct
  source 1..27: mol_type = other DNA
acaagtaagcaccagacttaccgacga

SEQ ID NO: 54 - DNA, 26 bp, synthetic construct
  source 1..26: mol_type = other DNA
cctcgtcggtctttctggtgcttact

SEQ ID NO: 55 - DNA, 27 bp, synthetic construct
  source 1..27: mol_type = other DNA
acaagtaagcaccagaaagaccgacga

SEQ ID NO: 56 - DNA, 26 bp, synthetic construct
  source 1..26: mol_type = other DNA
cctcgtcggtatgtctggtgcttact

SEQ ID NO: 57 - DNA, 27 bp, synthetic construct
  source 1..27: mol_type = other DNA
acaagtaagcaccagacataccgacga

SEQ ID NO: 58 - DNA, 26 bp, synthetic construct
  source 1..26: mol_type = other DNA
cctcgtcggtaattctggtgcttact

SEQ ID NO: 59 - DNA, 27 bp, synthetic construct
  source 1..27: mol_type = other DNA
acaagtaagcaccagaattaccgacga

SEQ ID NO: 60 - DNA, 26 bp, synthetic construct
  source 1..26: mol_type = other DNA
cctcgtcggtccctctggtgcttact

SEQ ID NO: 61 - DNA, 27 bp, synthetic construct
  source 1..27: mol_type = other DNA
acaagtaagcaccagagggaccgacga

SEQ ID NO: 62 - DNA, 26 bp, synthetic construct
  source 1..26: mol_type = other DNA
cctcgtcggtcaatctggtgcttact

SEQ ID NO: 63 - DNA, 27 bp, synthetic construct
  source 1..27: mol_type = other DNA
acaagtaagcaccagattgaccgacga

SEQ ID NO: 64 - DNA, 26 bp, synthetic construct
  source 1..26: mol_type = other DNA
cctcgtcggtcgttctggtgcttact

SEQ ID NO: 65 - DNA, 27 bp, synthetic construct
  source 1..27: mol_type = other DNA
acaagtaagcaccagaacgaccgacga

SEQ ID NO: 66 - DNA, 26 bp, synthetic construct
  source 1..26: mol_type = other DNA
cctcgtcggtacctctggtgcttact

SEQ ID NO: 67 - DNA, 27 bp, synthetic construct
  source 1..27: mol_type = other DNA
acaagtaagcaccagaggtaccgacga

SEQ ID NO: 68 - DNA, 26 bp, synthetic construct
  source 1..26: mol_type = other DNA
cctcgtcggtgtgtctggtgcttact

SEQ ID NO: 69 - DNA, 27 bp, synthetic construct
  source 1..27: mol_type = other DNA
acaagtaagcaccagacacaccgacga

SEQ ID NO: 70 - DNA, 26 bp, synthetic construct
  source 1..26: mol_type = other DNA
cctcgtcggttggtctggtgcttact

SEQ ID NO: 71 - DNA, 27 bp, synthetic construct
  source 1..27: mol_type = other DNA
acaagtaagcaccagaccaaccgacga

SEQ ID NO: 72 - DNA, 26 bp, synthetic construct
  source 1..26: mol_type = other DNA
cctcgtcggttactctggtgcttact

SEQ ID NO: 73 - DNA, 27 bp, synthetic construct
  source 1..27: mol_type = other DNA
acaagtaagcaccagagtaaccgacga

SEQ ID NO: 74 - protein, 499 aa, synthetic construct
MNSFILATEVTNPDVSQDLLDWTDRISTLAYLVAALLFILALAGLSKQQSASRGNTFGIAGMTIALVATVFKAAVQSHADPENYNDAWVTILLVAVAMLIGAVIGIARASKVEMTGMPELIAMLHCFVGAAAVLIGVNSFIHAEHTSEAGYEKFHLGEVYLGIFIGAVTFTGSIIAYLKLSARMKGAPLTLPGRNLLNLAIIVLSVVGMVFFILTGTEEADNKAVAWTILGIMIVLALLLGLHLVAAIGGGDMPVVVSMLNSYSGWAAAAAGFMLANPLLIITGALVGASGAYLSYIMCKAMNRSFISVILGGFGTEASSSDDRDYGTHTEITAEETAELLKGAKSVMITPGYGMAVAQAQYPVAAMVSKLREKGVDVTFGIHPVAGRLPGHMNVLLAEAKVPYDIVHEMDEVNDDFADIDVVLVIGANDTVNPIAEEPGSPLAGMPVLKVWEAKRVVVFKRSMGAGYAGVQNPLFFNENTDMLLGDAKDSVEKITSAL

SEQ ID NO: 75 - DNA, 1500 bp, synthetic construct
  source 1..1500: mol_type = other DNA
atgaactcttttattctggcgaccgaagtgaccaaccccgatgtgtctcaggatttgctggactggaccgaccgtatttctaccctcgcttaccttgtggcagccctgctcttcatcctcgctttggcgggtctgtctaagcagcaatccgctgcgcgcggcaacaccttcggtatcgctggtatgaccattgcgctcgttgcaaccgtgtttaaagcagccgtgcagtcccacgcagatccagagaactataatgacgcatgggtcaccatcttgcttgtcgcagttgccatgctgattggtgcagtcatcggcattgctcgcgcgtccaaggttgagatgaccggtatgccagaactcatcgccatgttgcactgcttcgtgggtgctgcggcagtgctgatcggcgtcaactcttttattcacgcggaacacacctccgaggcaggttacgaaaaattccaccttggcgaagtgtatctgggtatcttcattggcgcagtcacctttaccggctctatcattgcctaccttaagctgtccgcccgcatgaaaggtgctccgctcaccttgcccggccgtaacctgctcaatctcgcaatcattgtgttgtccgtggtcggtatggtcttctttatcctgaccggcaccgaagaggcagataacaaggcagttgcctggaccattcttggtatcatgattgtgctggccttgcttctgggtcttcacctggtcgcagctatcggtggtggtgacatgccggttgtggtctccatgctcaactcttactccggttgggcggcagccgctgcgggcttcatgttggctaatcccctcttgatcattaccggcgccctcgtcggtgcatctggtgcttacttgtcctatatcatgtgtaaggctatgaaccgctctttcatctccgttattctgggtggctttggcaccgaagcgtcctcttccgatgaccgtgattatggcacccacaccgaggtcaccgcggaagagaccgcagaacttctgaagaacgccaaatccgttatgatcacccctggttacggtatggctgtggcacaggcacaatatcccgttgcagcaatggtgtccaagctgcgcgagaagggtgtggacgtcaccttcggcatccacccagtcgcaggtcgtctccctggccacatgaacgttctcttggccgaagctaaggtcccgtacgatattgttcacgaaatggacgaagtgaatgatgactttgccgacatcgacgttgtgctcgttattggcgccaacgataccgtgaatccaatcgctgaagagccaggttctcctattgcgggtatgccagtcttgaaggtttgggacgcaaaccgcgtcgttgtgttcaaacgctctatgggcgccggctacgctggcgttcaaaacccattgttctttaacgagaacaccgatatgcttctgggcgatgctaaggactctgtggaaaaaatcacctccgcgctgtaa

SEQ ID NO: 76 - protein, 499 aa, synthetic construct
MNSFILATEVTNPDVSQDLLDWTDRISTLAYLVAALLFILALAGLSKQQSASRGNTFGIAGMTIALVATVFKAAVQSHADPENYNDAWVTILLVAVAMLIGAVIGIARASKVEMTGMPELIAMLHCFVGAAAVLIGVNSFIHAEHTSEAGYEKFHLGEVYLGIFIGAVTFTGSIIAYLKLSARMKGAPLTLPGRNLLNLAIIVLSVVGMVFFILTGTEEADNKAVAWTILGIMIVLALLLGLHLVAAIGGGDMPVVVSMLNSYSGWAAAAAGFMLANPLLIITGALVGCSGAYLSYIMCKAMNRSFISVILGGFGTEASSSDDRDYGTHTEITAEETAELLKGAKSVMITPGYGMAVAQAQYPVAAMVSKLREKGVDVTFGIHPVAGRLPGHMNVLLAEAKVPYDIVHEMDEVNDDFADIDVVLVIGANDTVNPIAEEPGSPLAGMPVLKVWEAKRVVVFKRSMGAGYAGVQNPLFFNENTDMLLGDAKDSVEKITSAL

SEQ ID NO: 77 - DNA, 1500 bp, synthetic construct
  source 1..1500: mol_type = other DNA
atgaactcttttattctggcgaccgaagtgaccaaccccgatgtgtctcaggatttgctggactggaccgaccgtatttctaccctcgcttaccttgtggcagccctgctcttcatcctcgctttggcgggtctgtctaagcagcaatccgctgcgcgcggcaacaccttcggtatcgctggtatgaccattgcgctcgttgcaaccgtgtttaaagcagccgtgcagtcccacgcagatccagagaactataatgacgcatgggtcaccatcttgcttgtcgcagttgccatgctgattggtgcagtcatcggcattgctcgcgcgtccaaggttgagatgaccggtatgccagaactcatcgccatgttgcactgcttcgtgggtgctgcggcagtgctgatcggcgtcaactcttttattcacgcggaacacacctccgaggcaggttacgaaaaattccaccttggcgaagtgtatctgggtatcttcattggcgcagtcacctttaccggctctatcattgcctaccttaagctgtccgcccgcatgaaaggtgctccgctcaccttgcccggccgtaacctgctcaatctcgcaatcattgtgttgtccgtggtcggtatggtcttctttatcctgaccggcaccgaagaggcagataacaaggcagttgcctggaccattcttggtatcatgattgtgctggccttgcttctgggtcttcacctggtcgcagctatcggtggtggtgacatgccggttgtggtctccatgctcaactcttactccggttgggcggcagccgctgcgggcttcatgttggctaatcccctcttgatcattaccggcgccctcgtcggttgctctggtgcttacttgtcctatatcatgtgtaaggctatgaaccgctctttcatctccgttattctgggtggctttggcaccgaagcgtcctcttccgatgaccgtgattatggcacccacaccgaggtcaccgcggaagagaccgcagaacttctgaagaacgccaaatccgttatgatcacccctggttacggtatggctgtggcacaggcacaatatcccgttgcagcaatggtgtccaagctgcgcgagaagggtgtggacgtcaccttcggcatccacccagtcgcaggtcgtctccctggccacatgaacgttctcttggccgaagctaaggtcccgtacgatattgttcacgaaatggacgaagtgaatgatgactttgccgacatcgacgttgtgctcgttattggcgccaacgataccgtgaatccaatcgctgaagagccaggttctcctattgcgggtatgccagtcttgaaggtttgggacgcaaaccgcgtcgttgtgttcaaacgctctatgggcgccggctacgctggcgttcaaaacccattgttctttaacgagaacaccgatatgcttctgggcgatgctaaggactctgtggaaaaaatcacctccgcgctgtaa

SEQ ID NO: 78 - protein, 499 aa, synthetic construct
MNSFILATEVTNPDVSQDLLDWTDRISTLAYLVAALLFILALAGLSKQQSASRGNTFGIAGMTIALVATVFKAAVQSHADPENYNDAWVTILLVAVAMLIGAVIGIARASKVEMTGMPELIAMLHCFVGAAAVLIGVNSFIHAEHTSEAGYEKFHLGEVYLGIFIGAVTFTGSIIAYLKLSARMKGAPLTLPGRNLLNLAIIVLSVVGMVFFILTGTEEADNKAVAWTILGIMIVLALLLGLHLVAAIGGGDMPVVVSMLNSYSGWAAAAAGFMLANPLLIITGALVGISGAYLSYIMCKAMNRSFISVILGGFGTEASSSDDRDYGTHTEITAEETAELLKGAKSVMITPGYGMAVAQAQYPVAAMVSKLREKGVDVTFGIHPVAGRLPGHMNVLLAEAKVPYDIVHEMDEVNDDFADIDVVLVIGANDTVNPIAEEPGSPLAGMPVLKVWEAKRVVVFKRSMGAGYAGVQNPLFFNENTDMLLGDAKDSVEKITSAL

SEQ ID NO: 79 - DNA, 1500 bp, synthetic construct
  source 1..1500: mol_type = other DNA
atgaactcttttattctggcgaccgaagtgaccaaccccgatgtgtctcaggatttgctggactggaccgaccgtatttctaccctcgcttaccttgtggcagccctgctcttcatcctcgctttggcgggtctgtctaagcagcaatccgctgcgcgcggcaacaccttcggtatcgctggtatgaccattgcgctcgttgcaaccgtgtttaaagcagccgtgcagtcccacgcagatccagagaactataatgacgcatgggtcaccatcttgcttgtcgcagttgccatgctgattggtgcagtcatcggcattgctcgcgcgtccaaggttgagatgaccggtatgccagaactcatcgccatgttgcactgcttcgtgggtgctgcggcagtgctgatcggcgtcaactcttttattcacgcggaacacacctccgaggcaggttacgaaaaattccaccttggcgaagtgtatctgggtatcttcattggcgcagtcacctttaccggctctatcattgcctaccttaagctgtccgcccgcatgaaaggtgctccgctcaccttgcccggccgtaacctgctcaatctcgcaatcattgtgttgtccgtggtcggtatggtcttctttatcctgaccggcaccgaagaggcagataacaaggcagttgcctggaccattcttggtatcatgattgtgctggccttgcttctgggtcttcacctggtcgcagctatcggtggtggtgacatgccggttgtggtctccatgctcaactcttactccggttgggcggcagccgctgcgggcttcatgttggctaatcccctcttgatcattaccggcgccctcgtcggtatctctggtgcttacttgtcctatatcatgtgtaaggctatgaaccgctctttcatctccgttattctgggtggctttggcaccgaagcgtcctcttccgatgaccgtgattatggcacccacaccgaggtcaccgcggaagagaccgcagaacttctgaagaacgccaaatccgttatgatcacccctggttacggtatggctgtggcacaggcacaatatcccgttgcagcaatggtgtccaagctgcgcgagaagggtgtggacgtcaccttcggcatccacccagtcgcaggtcgtctccctggccacatgaacgttctcttggccgaagctaaggtcccgtacgatattgttcacgaaatggacgaagtgaatgatgactttgccgacatcgacgttgtgctcgttattggcgccaacgataccgtgaatccaatcgctgaagagccaggttctcctattgcgggtatgccagtcttgaaggtttgggacgcaaaccgcgtcgttgtgttcaaacgctctatgggcgccggctacgctggcgttcaaaacccattgttctttaacgagaacaccgatatgcttctgggcgatgctaaggactctgtggaaaaaatcacctccgcgctgtaa

SEQ ID NO: 80 - protein, 499 aa, synthetic construct
MNSFILATEVTNPDVSQDLLDWTDRISTLAYLVAALLFILALAGLSKQQSASRGNTFGIAGMTIALVATVFKAAVQSHADPENYNDAWVTILLVAVAMLIGAVIGIARASKVEMTGMPELIAMLHCFVGAAAVLIGVNSFIHAEHTSEAGYEKFHLGEVYLGIFIGAVTFTGSIIAYLKLSARMKGAPLTLPGRNLLNLAIIVLSVVGMVFFILTGTEEADNKAVAWTILGIMIVLALLLGLHLVAAIGGGDMPVVVSMLNSYSGWAAAAAGFMLANPLLIITGALVGMSGAYLSYIMCKAMNRSFISVILGGFGTEASSSDDRDYGTHTEITAEETAELLKGAKSVMITPGYGMAVAQAQYPVAAMVSKLREKGVDVTFGIHPVAGRLPGHMNVLLAEAKVPYDIVHEMDEVNDDFADIDVVLVIGANDTVNPIAEEPGSPLAGMPVLKVWEAKRVVVFKRSMGAGYAGVQNPLFFNENTDMLLGDAKDSVEKITSAL

SEQ ID NO: 81 - DNA, 1500 bp, synthetic construct
  source 1..1500: mol_type = other DNA
atgaactcttttattctggcgaccgaagtgaccaaccccgatgtgtctcaggatttgctggactggaccgaccgtatttctaccctcgcttaccttgtggcagccctgctcttcatcctcgctttggcgggtctgtctaagcagcaatccgctgcgcgcggcaacaccttcggtatcgctggtatgaccattgcgctcgttgcaaccgtgtttaaagcagccgtgcagtcccacgcagatccagagaactataatgacgcatgggtcaccatcttgcttgtcgcagttgccatgctgattggtgcagtcatcggcattgctcgcgcgtccaaggttgagatgaccggtatgccagaactcatcgccatgttgcactgcttcgtgggtgctgcggcagtgctgatcggcgtcaactcttttattcacgcggaacacacctccgaggcaggttacgaaaaattccaccttggcgaagtgtatctgggtatcttcattggcgcagtcacctttaccggctctatcattgcctaccttaagctgtccgcccgcatgaaaggtgctccgctcaccttgcccggccgtaacctgctcaatctcgcaatcattgtgttgtccgtggtcggtatggtcttctttatcctgaccggcaccgaagaggcagataacaaggcagttgcctggaccattcttggtatcatgattgtgctggccttgcttctgggtcttcacctggtcgcagctatcggtggtggtgacatgccggttgtggtctccatgctcaactcttactccggttgggcggcagccgctgcgggcttcatgttggctaatcccctcttgatcattaccggcgccctcgtcggtatgtctggtgcttacttgtcctatatcatgtgtaaggctatgaaccgctctttcatctccgttattctgggtggctttggcaccgaagcgtcctcttccgatgaccgtgattatggcacccacaccgaggtcaccgcggaagagaccgcagaacttctgaagaacgccaaatccgttatgatcacccctggttacggtatggctgtggcacaggcacaatatcccgttgcagcaatggtgtccaagctgcgcgagaagggtgtggacgtcaccttcggcatccacccagtcgcaggtcgtctccctggccacatgaacgttctcttggccgaagctaaggtcccgtacgatattgttcacgaaatggacgaagtgaatgatgactttgccgacatcgacgttgtgctcgttattggcgccaacgataccgtgaatccaatcgctgaagagccaggttctcctattgcgggtatgccagtcttgaaggtttgggacgcaaaccgcgtcgttgtgttcaaacgctctatgggcgccggctacgctggcgttcaaaacccattgttctttaacgagaacaccgatatgcttctgggcgatgctaaggactctgtggaaaaaatcacctccgcgctgtaa

SEQ ID NO: 82 - protein, 499 aa, synthetic construct
MNSFILATEVTNPDVSQDLLDWTDRISTLAYLVAALLFILALAGLSKQQSASRGNTFGIAGMTIALVATVFKAAVQSHADPENYNDAWVTILLVAVAMLIGAVIGIARASKVEMTGMPELIAMLHCFVGAAAVLIGVNSFIHAEHTSEAGYEKFHLGEVYLGIFIGAVTFTGSIIAYLKLSARMKGAPLTLPGRNLLNLAIIVLSVVGMVFFILTGTEEADNKAVAWTILGIMIVLALLLGLHLVAAIGGGDMPVVVSMLNSYSGWAAAAAGFMLANPLLIITGALVGTSGAYLSYIMCKAMNRSFISVILGGFGTEASSSDDRDYGTHTEITAEETAELLKGAKSVMITPGYGMAVAQAQYPVAAMVSKLREKGVDVTFGIHPVAGRLPGHMNVLLAEAKVPYDIVHEMDEVNDDFADIDVVLVIGANDTVNPIAEEPGSPLAGMPVLKVWEAKRVVVFKRSMGAGYAGVQNPLFFNENTDMLLGDAKDSVEKITSAL

SEQ ID NO: 83 - DNA, 1500 bp, synthetic construct
  source 1..1500: mol_type = other DNA
atgaactcttttattctggcgaccgaagtgaccaaccccgatgtgtctcaggatttgctggactggaccgaccgtatttctaccctcgcttaccttgtggcagccctgctcttcatcctcgctttggcgggtctgtctaagcagcaatccgctgcgcgcggcaacaccttcggtatcgctggtatgaccattgcgctcgttgcaaccgtgtttaaagcagccgtgcagtcccacgcagatccagagaactataatgacgcatgggtcaccatcttgcttgtcgcagttgccatgctgattggtgcagtcatcggcattgctcgcgcgtccaaggttgagatgaccggtatgccagaactcatcgccatgttgcactgcttcgtgggtgctgcggcagtgctgatcggcgtcaactcttttattcacgcggaacacacctccgaggcaggttacgaaaaattccaccttggcgaagtgtatctgggtatcttcattggcgcagtcacctttaccggctctatcattgcctaccttaagctgtccgcccgcatgaaaggtgctccgctcaccttgcccggccgtaacctgctcaatctcgcaatcattgtgttgtccgtggtcggtatggtcttctttatcctgaccggcaccgaagaggcagataacaaggcagttgcctggaccattcttggtatcatgattgtgctggccttgcttctgggtcttcacctggtcgcagctatcggtggtggtgacatgccggttgtggtctccatgctcaactcttactccggttgggcggcagccgctgcgggcttcatgttggctaatcccctcttgatcattaccggcgccctcgtcggtacctctggtgcttacttgtcctatatcatgtgtaaggctatgaaccgctctttcatctccgttattctgggtggctttggcaccgaagcgtcctcttccgatgaccgtgattatggcacccacaccgaggtcaccgcggaagagaccgcagaacttctgaagaacgccaaatccgttatgatcacccctggttacggtatggctgtggcacaggcacaatatcccgttgcagcaatggtgtccaagctgcgcgagaagggtgtggacgtcaccttcggcatccacccagtcgcaggtcgtctccctggccacatgaacgttctcttggccgaagctaaggtcccgtacgatattgttcacgaaatggacgaagtgaatgatgactttgccgacatcgacgttgtgctcgttattggcgccaacgataccgtgaatccaatcgctgaagagccaggttctcctattgcgggtatgccagtcttgaaggtttgggacgcaaaccgcgtcgttgtgttcaaacgctctatgggcgccggctacgctggcgttcaaaacccattgttctttaacgagaacaccgatatgcttctgggcgatgctaaggactctgtggaaaaaatcacctccgcgctgtaa

SEQ ID NO: 84 - protein, 499 aa, synthetic construct
MNSFILATEVTNPDVSQDLLDWTDRISTLAYLVAALLFILALAGLSKQQSASRGNTFGIAGMTIALVATVFKAAVQSHADPENYNDAWVTILLVAVAMLIGAVIGIARASKVEMTGMPELIAMLHCFVGAAAVLIGVNSFIHAEHTSEAGYEKFHLGEVYLGIFIGAVTFTGSIIAYLKLSARMKGAPLTLPGRNLLNLAIIVLSVVGMVFFILTGTEEADNKAVAWTILGIMIVLALLLGLHLVAAIGGGDMPVVVSMLNSYSGWAAAAAGFMLANPLLIITGALVGDSGAYLSYIMCKAMNRSFISVILGGFGTEASSSDDRDYGTHTEITAEETAELLKGAKSVMITPGYGMAVAQAQYPVAAMVSKLREKGVDVTFGIHPVAGRLPGHMNVLLAEAKVPYDIVHEMDEVNDDFADIDVVLVIGANDTVNPIAEEPGSPLAGMPVLKVWEAKRVVVFKRSMGAGYAGVQNPLFFNENTDMLLGDAKDSVEKITSAL

SEQ ID NO: 85 - DNA, 1500 bp, synthetic construct
  source 1..1500: mol_type = other DNA
atgaactcttttattctggcgaccgaagtgaccaaccccgatgtgtctcaggatttgctggactggaccgaccgtatttctaccctcgcttaccttgtggcagccctgctcttcatcctcgctttggcgggtctgtctaagcagcaatccgctgcgcgcggcaacaccttcggtatcgctggtatgaccattgcgctcgttgcaaccgtgtttaaagcagccgtgcagtcccacgcagatccagagaactataatgacgcatgggtcaccatcttgcttgtcgcagttgccatgctgattggtgcagtcatcggcattgctcgcgcgtccaaggttgagatgaccggtatgccagaactcatcgccatgttgcactgcttcgtgggtgctgcggcagtgctgatcggcgtcaactcttttattcacgcggaacacacctccgaggcaggttacgaaaaattccaccttggcgaagtgtatctgggtatcttcattggcgcagtcacctttaccggctctatcattgcctaccttaagctgtccgcccgcatgaaaggtgctccgctcaccttgcccggccgtaacctgctcaatctcgcaatcattgtgttgtccgtggtcggtatggtcttctttatcctgaccggcaccgaagaggcagataacaaggcagttgcctggaccattcttggtatcatgattgtgctggccttgcttctgggtcttcacctggtcgcagctatcggtggtggtgacatgccggttgtggtctccatgctcaactcttactccggttgggcggcagccgctgcgggcttcatgttggctaatcccctcttgatcattaccggcgccctcgtcggtgattctggtgcttacttgtcctatatcatgtgtaaggctatgaaccgctctttcatctccgttattctgggtggctttggcaccgaagcgtcctcttccgatgaccgtgattatggcacccacaccgaggtcaccgcggaagagaccgcagaacttctgaagaacgccaaatccgttatgatcacccctggttacggtatggctgtggcacaggcacaatatcccgttgcagcaatggtgtccaagctgcgcgagaagggtgtggacgtcaccttcggcatccacccagtcgcaggtcgtctccctggccacatgaacgttctcttggccgaagctaaggtcccgtacgatattgttcacgaaatggacgaagtgaatgatgactttgccgacatcgacgttgtgctcgttattggcgccaacgataccgtgaatccaatcgctgaagagccaggttctcctattgcgggtatgccagtcttgaaggtttgggacgcaaaccgcgtcgttgtgttcaaacgctctatgggcgccggctacgctggcgttcaaaacccattgttctttaacgagaacaccgatatgcttctgggcgatgctaaggactctgtggaaaaaatcacctccgcgctgtaa

SEQ ID NO: 86 - protein, 499 aa, synthetic construct
MNSFILATEVTNPDVSQDLLDWTDRISTLAYLVAALLFILALAGLSKQQSASRGNTFGIAGMTIALVATVFKAAVQSHADPENYNDAWVTILLVAVAMLIGAVIGIARASKVEMTGMPELIAMLHCFVGAAAVLIGVNSFIHAEHTSEAGYEKFHLGEVYLGIFIGAVTFTGSIIAYLKLSARMKGAPLTLPGRNLLNLAIIVLSVVGMVFFILTGTEEADNKAVAWTILGIMIVLALLLGLHLVAAIGGGDMPVVVSMLNSYSGWAAAAAGFMLANPLLIITGALVGESGAYLSYIMCKAMNRSFISVILGGFGTEASSSDDRDYGTHTEITAEETAELLKGAKSVMITPGYGMAVAQAQYPVAAMVSKLREKGVDVTFGIHPVAGRLPGHMNVLLAEAKVPYDIVHEMDEVNDDFADIDVVLVIGANDTVNPIAEEPGSPLAGMPVLKVWEAKRVVVFKRSMGAGYAGVQNPLFFNENTDMLLGDAKDSVEKITSAL

SEQ ID NO: 87 - DNA, 1500 bp, synthetic construct
  source 1..1500: mol_type = other DNA
atgaactcttttattctggcgaccgaagtgaccaaccccgatgtgtctcaggatttgctggactggaccgaccgtatttctaccctcgcttaccttgtggcagccctgctcttcatcctcgctttggcgggtctgtctaagcagcaatccgctgcgcgcggcaacaccttcggtatcgctggtatgaccattgcgctcgttgcaaccgtgtttaaagcagccgtgcagtcccacgcagatccagagaactataatgacgcatgggtcaccatcttgcttgtcgcagttgccatgctgattggtgcagtcatcggcattgctcgcgcgtccaaggttgagatgaccggtatgccagaactcatcgccatgttgcactgcttcgtgggtgctgcggcagtgctgatcggcgtcaactcttttattcacgcggaacacacctccgaggcaggttacgaaaaattccaccttggcgaagtgtatctgggtatcttcattggcgcagtcacctttaccggctctatcattgcctaccttaagctgtccgcccgcatgaaaggtgctccgctcaccttgcccggccgtaacctgctcaatctcgcaatcattgtgttgtccgtggtcggtatggtcttctttatcctgaccggcaccgaagaggcagataacaaggcagttgcctggaccattcttggtatcatgattgtgctggccttgcttctgggtcttcacctggtcgcagctatcggtggtggtgacatgccggttgtggtctccatgctcaactcttactccggttgggcggcagccgctgcgggcttcatgttggctaatcccctcttgatcattaccggcgccctcgtcggtgaatctggtgcttacttgtcctatatcatgtgtaaggctatgaaccgctctttcatctccgttattctgggtggctttggcaccgaagcgtcctcttccgatgaccgtgattatggcacccacaccgaggtcaccgcggaagagaccgcagaacttctgaagaacgccaaatccgttatgatcacccctggttacggtatggctgtggcacaggcacaatatcccgttgcagcaatggtgtccaagctgcgcgagaagggtgtggacgtcaccttcggcatccacccagtcgcaggtcgtctccctggccacatgaacgttctcttggccgaagctaaggtcccgtacgatattgttcacgaaatggacgaagtgaatgatgactttgccgacatcgacgttgtgctcgttattggcgccaacgataccgtgaatccaatcgctgaagagccaggttctcctattgcgggtatgccagtcttgaaggtttgggacgcaaaccgcgtcgttgtgttcaaacgctctatgggcgccggctacgctggcgttcaaaacccattgttctttaacgagaacaccgatatgcttctgggcgatgctaaggactctgtggaaaaaatcacctccgcgctgtaa

SEQ ID NO: 88 - protein, 499 aa, synthetic construct
MNSFILATEVTNPDVSQDLLDWTDRISTLAYLVAALLFILALAGLSKQQSASRGNTFGIAGMTIALVATVFKAAVQSHADPENYNDAWVTILLVAVAMLIGAVIGIARASKVEMTGMPELIAMLHCFVGAAAVLIGVNSFIHAEHTSEAGYEKFHLGEVYLGIFIGAVTFTGSIIAYLKLSARMKGAPLTLPGRNLLNLAIIVLSVVGMVFFILTGTEEADNKAVAWTILGIMIVLALLLGLHLVAAIGGGDMPVVVSMLNSYSGWAAAAAGFMLANPLLIITGALVGFSGAYLSYIMCKAMNRSFISVILGGFGTEASSSDDRDYGTHTEITAEETAELLKGAKSVMITPGYGMAVAQAQYPVAAMVSKLREKGVDVTFGIHPVAGRLPGHMNVLLAEAKVPYDIVHEMDEVNDDFADIDVVLVIGANDTVNPIAEEPGSPLAGMPVLKVWEAKRVVVFKRSMGAGYAGVQNPLFFNENTDMLLGDAKDSVEKITSAL

SEQ ID NO: 89 - DNA, 1500 bp, synthetic construct
  source 1..1500: mol_type = other DNA
atgaactcttttattctggcgaccgaagtgaccaaccccgatgtgtctcaggatttgctggactggaccgaccgtatttctaccctcgcttaccttgtggcagccctgctcttcatcctcgctttggcgggtctgtctaagcagcaatccgctgcgcgcggcaacaccttcggtatcgctggtatgaccattgcgctcgttgcaaccgtgtttaaagcagccgtgcagtcccacgcagatccagagaactataatgacgcatgggtcaccatcttgcttgtcgcagttgccatgctgattggtgcagtcatcggcattgctcgcgcgtccaaggttgagatgaccggtatgccagaactcatcgccatgttgcactgcttcgtgggtgctgcggcagtgctgatcggcgtcaactcttttattcacgcggaacacacctccgaggcaggttacgaaaaattccaccttggcgaagtgtatctgggtatcttcattggcgcagtcacctttaccggctctatcattgcctaccttaagctgtccgcccgcatgaaaggtgctccgctcaccttgcccggccgtaacctgctcaatctcgcaatcattgtgttgtccgtggtcggtatggtcttctttatcctgaccggcaccgaagaggcagataacaaggcagttgcctggaccattcttggtatcatgattgtgctggccttgcttctgggtcttcacctggtcgcagctatcggtggtggtgacatgccggttgtggtctccatgctcaactcttactccggttgggcggcagccgctgcgggcttcatgttggctaatcccctcttgatcattaccggcgccctcgtcggtttctctggtgcttacttgtcctatatcatgtgtaaggctatgaaccgctctttcatctccgttattctgggtggctttggcaccgaagcgtcctcttccgatgaccgtgattatggcacccacaccgaggtcaccgcggaagagaccgcagaacttctgaagaacgccaaatccgttatgatcacccctggttacggtatggctgtggcacaggcacaatatcccgttgcagcaatggtgtccaagctgcgcgagaagggtgtggacgtcaccttcggcatccacccagtcgcaggtcgtctccctggccacatgaacgttctcttggccgaagctaaggtcccgtacgatattgttcacgaaatggacgaagtgaatgatgactttgccgacatcgacgttgtgctcgttattggcgccaacgataccgtgaatccaatcgctgaagagccaggttctcctattgcgggtatgccagtcttgaaggtttgggacgcaaaccgcgtcgttgtgttcaaacgctctatgggcgccggctacgctggcgttcaaaacccattgttctttaacgagaacaccgatatgcttctgggcgatgctaaggactctgtggaaaaaatcacctccgcgctgtaa

SEQ ID NO: 90 - protein, 499 aa, synthetic construct
MNSFILATEVTNPDVSQDLLDWTDRISTLAYLVAALLFILALAGLSKQQSASRGNTFGIAGMTIALVATVFKAAVQSHADPENYNDAWVTILLVAVAMLIGAVIGIARASKVEMTGMPELIAMLHCFVGAAAVLIGVNSFIHAEHTSEAGYEKFHLGEVYLGIFIGAVTFTGSIIAYLKLSARMKGAPLTLPGRNLLNLAIIVLSVVGMVFFILTGTEEADNKAVAWTILGIMIVLALLLGLHLVAAIGGGDMPVVVSMLNSYSGWAAAAAGFMLANPLLIITGALVGGSGAYLSYIMCKAMNRSFISVILGGFGTEASSSDDRDYGTHTEITAEETAELLKGAKSVMITPGYGMAVAQAQYPVAAMVSKLREKGVDVTFGIHPVAGRLPGHMNVLLAEAKVPYDIVHEMDEVNDDFADIDVVLVIGANDTVNPIAEEPGSPLAGMPVLKVWEAKRVVVFKRSMGAGYAGVQNPLFFNENTDMLLGDAKDSVEKITSAL

SEQ ID NO: 91 - DNA, 1500 bp, synthetic construct
  source 1..1500: mol_type = other DNA
atgaactcttttattctggcgaccgaagtgaccaaccccgatgtgtctcaggatttgctggactggaccgaccgtatttctaccctcgcttaccttgtggcagccctgctcttcatcctcgctttggcgggtctgtctaagcagcaatccgctgcgcgcggcaacaccttcggtatcgctggtatgaccattgcgctcgttgcaaccgtgtttaaagcagccgtgcagtcccacgcagatccagagaactataatgacgcatgggtcaccatcttgcttgtcgcagttgccatgctgattggtgcagtcatcggcattgctcgcgcgtccaaggttgagatgaccggtatgccagaactcatcgccatgttgcactgcttcgtgggtgctgcggcagtgctgatcggcgtcaactcttttattcacgcggaacacacctccgaggcaggttacgaaaaattccaccttggcgaagtgtatctgggtatcttcattggcgcagtcacctttaccggctctatcattgcctaccttaagctgtccgcccgcatgaaaggtgctccgctcaccttgcccggccgtaacctgctcaatctcgcaatcattgtgttgtccgtggtcggtatggtcttctttatcctgaccggcaccgaagaggcagataacaaggcagttgcctggaccattcttggtatcatgattgtgctggccttgcttctgggtcttcacctggtcgcagctatcggtggtggtgacatgccggttgtggtctccatgctcaactcttactccggttgggcggcagccgctgcgggcttcatgttggctaatcccctcttgatcattaccggcgccctcgtcggtggctctggtgcttacttgtcctatatcatgtgtaaggctatgaaccgctctttcatctccgttattctgggtggctttggcaccgaagcgtcctcttccgatgaccgtgattatggcacccacaccgaggtcaccgcggaagagaccgcagaacttctgaagaacgccaaatccgttatgatcacccctggttacggtatggctgtggcacaggcacaatatcccgttgcagcaatggtgtccaagctgcgcgagaagggtgtggacgtcaccttcggcatccacccagtcgcaggtcgtctccctggccacatgaacgttctcttggccgaagctaaggtcccgtacgatattgttcacgaaatggacgaagtgaatgatgactttgccgacatcgacgttgtgctcgttattggcgccaacgataccgtgaatccaatcgctgaagagccaggttctcctattgcgggtatgccagtcttgaaggtttgggacgcaaaccgcgtcgttgtgttcaaacgctctatgggcgccggctacgctggcgttcaaaacccattgttctttaacgagaacaccgatatgcttctgggcgatgctaaggactctgtggaaaaaatcacctccgcgctgtaa

SEQ ID NO: 92 - protein, 499 aa, synthetic construct
MNSFILATEVTNPDVSQDLLDWTDRISTLAYLVAALLFILALAGLSKQQSASRGNTFGIAGMTIALVATVFKAAVQSHADPENYNDAWVTILLVAVAMLIGAVIGIARASKVEMTGMPELIAMLHCFVGAAAVLIGVNSFIHAEHTSEAGYEKFHLGEVYLGIFIGAVTFTGSIIAYLKLSARMKGAPLTLPGRNLLNLAIIVLSVVGMVFFILTGTEEADNKAVAWTILGIMIVLALLLGLHLVAAIGGGDMPVVVSMLNSYSGWAAAAAGFMLANPLLIITGALVGHSGAYLSYIMCKAMNRSFISVILGGFGTEASSSDDRDYGTHTEITAEETAELLKGAKSVMITPGYGMAVAQAQYPVAAMVSKLREKGVDVTFGIHPVAGRLPGHMNVLLAEAKVPYDIVHEMDEVNDDFADIDVVLVIGANDTVNPIAEEPGSPLAGMPVLKVWEAKRVVVFKRSMGAGYAGVQNPLFFNENTDMLLGDAKDSVEKITSAL

SEQ ID NO: 93 - DNA, 1500 bp, synthetic construct
  source 1..1500: mol_type = other DNA
atgaactcttttattctggcgaccgaagtgaccaaccccgatgtgtctcaggatttgctggactggaccgaccgtatttctaccctcgcttaccttgtggcagccctgctcttcatcctcgctttggcgggtctgtctaagcagcaatccgctgcgcgcggcaacaccttcggtatcgctggtatgaccattgcgctcgttgcaaccgtgtttaaagcagccgtgcagtcccacgcagatccagagaactataatgacgcatgggtcaccatcttgcttgtcgcagttgccatgctgattggtgcagtcatcggcattgctcgcgcgtccaaggttgagatgaccggtatgccagaactcatcgccatgttgcactgcttcgtgggtgctgcggcagtgctgatcggcgtcaactcttttattcacgcggaacacacctccgaggcaggttacgaaaaattccaccttggcgaagtgtatctgggtatcttcattggcgcagtcacctttaccggctctatcattgcctaccttaagctgtccgcccgcatgaaaggtgctccgctcaccttgcccggccgtaacctgctcaatctcgcaatcattgtgttgtccgtggtcggtatggtcttctttatcctgaccggcaccgaagaggcagataacaaggcagttgcctggaccattcttggtatcatgattgtgctggccttgcttctgggtcttcacctggtcgcagctatcggtggtggtgacatgccggttgtggtctccatgctcaactcttactccggttgggcggcagccgctgcgggcttcatgttggctaatcccctcttgatcattaccggcgccctcgtcggtcactctggtgcttacttgtcctatatcatgtgtaaggctatgaaccgctctttcatctccgttattctgggtggctttggcaccgaagcgtcctcttccgatgaccgtgattatggcacccacaccgaggtcaccgcggaagagaccgcagaacttctgaagaacgccaaatccgttatgatcacccctggttacggtatggctgtggcacaggcacaatatcccgttgcagcaatggtgtccaagctgcgcgagaagggtgtggacgtcaccttcggcatccacccagtcgcaggtcgtctccctggccacatgaacgttctcttggccgaagctaaggtcccgtacgatattgttcacgaaatggacgaagtgaatgatgactttgccgacatcgacgttgtgctcgttattggcgccaacgataccgtgaatccaatcgctgaagagccaggttctcctattgcgggtatgccagtcttgaaggtttgggacgcaaaccgcgtcgttgtgttcaaacgctctatgggcgccggctacgctggcgttcaaaacccattgttctttaacgagaacaccgatatgcttctgggcgatgctaaggactctgtggaaaaaatcacctccgcgctgtaa

SEQ ID NO: 94 - protein, 499 aa, synthetic construct
MNSFILATEVTNPDVSQDLLDWTDRISTLAYLVAALLFILALAGLSKQQSASRGNTFGIAGMTIALVATVFKAAVQSHADPENYNDAWVTILLVAVAMLIGAVIGIARASKVEMTGMPELIAMLHCFVGAAAVLIGVNSFIHAEHTSEAGYEKFHLGEVYLGIFIGAVTFTGSIIAYLKLSARMKGAPLTLPGRNLLNLAIIVLSVVGMVFFILTGTEEADNKAVAWTILGIMIVLALLLGLHLVAAIGGGDMPVVVSMLNSYSGWAAAAAGFMLANPLLIITGALVGKSGAYLSYIMCKAMNRSFISVILGGFGTEASSSDDRDYGTHTEITAEETAELLKGAKSVMITPGYGMAVAQAQYPVAAMVSKLREKGVDVTFGIHPVAGRLPGHMNVLLAEAKVPYDIVHEMDEVNDDFADIDVVLVIGANDTVNPIAEEPGSPLAGMPVLKVWEAKRVVVFKRSMGAGYAGVQNPLFFNENTDMLLGDAKDSVEKITSAL

SEQ ID NO: 95 - DNA, 1500 bp, synthetic construct
  source 1..1500: mol_type = other DNA
atgaactcttttattctggcgaccgaagtgaccaaccccgatgtgtctcaggatttgctggactggaccgaccgtatttctaccctcgcttaccttgtggcagccctgctcttcatcctcgctttggcgggtctgtctaagcagcaatccgctgcgcgcggcaacaccttcggtatcgctggtatgaccattgcgctcgttgcaaccgtgtttaaagcagccgtgcagtcccacgcagatccagagaactataatgacgcatgggtcaccatcttgcttgtcgcagttgccatgctgattggtgcagtcatcggcattgctcgcgcgtccaaggttgagatgaccggtatgccagaactcatcgccatgttgcactgcttcgtgggtgctgcggcagtgctgatcggcgtcaactcttttattcacgcggaacacacctccgaggcaggttacgaaaaattccaccttggcgaagtgtatctgggtatcttcattggcgcagtcacctttaccggctctatcattgcctaccttaagctgtccgcccgcatgaaaggtgctccgctcaccttgcccggccgtaacctgctcaatctcgcaatcattgtgttgtccgtggtcggtatggtcttctttatcctgaccggcaccgaagaggcagataacaaggcagttgcctggaccattcttggtatcatgattgtgctggccttgcttctgggtcttcacctggtcgcagctatcggtggtggtgacatgccggttgtggtctccatgctcaactcttactccggttgggcggcagccgctgcgggcttcatgttggctaatcccctcttgatcattaccggcgccctcgtcggtaagtctggtgcttacttgtcctatatcatgtgtaaggctatgaaccgctctttcatctccgttattctgggtggctttggcaccgaagcgtcctcttccgatgaccgtgattatggcacccacaccgaggtcaccgcggaagagaccgcagaacttctgaagaacgccaaatccgttatgatcacccctggttacggtatggctgtggcacaggcacaatatcccgttgcagcaatggtgtccaagctgcgcgagaagggtgtggacgtcaccttcggcatccacccagtcgcaggtcgtctccctggccacatgaacgttctcttggccgaagctaaggtcccgtacgatattgttcacgaaatggacgaagtgaatgatgactttgccgacatcgacgttgtgctcgttattggcgccaacgataccgtgaatccaatcgctgaagagccaggttctcctattgcgggtatgccagtcttgaaggtttgggacgcaaaccgcgtcgttgtgttcaaacgctctatgggcgccggctacgctggcgttcaaaacccattgttctttaacgagaacaccgatatgcttctgggcgatgctaaggactctgtggaaaaaatcacctccgcgctgtaa

SEQ ID NO: 96 - protein, 499 aa, synthetic construct
MNSFILATEVTNPDVSQDLLDWTDRISTLAYLVAALLFILALAGLSKQQSASRGNTFGIAGMTIALVATVFKAAVQSHADPENYNDAWVTILLVAVAMLIGAVIGIARASKVEMTGMPELIAMLHCFVGAAAVLIGVNSFIHAEHTSEAGYEKFHLGEVYLGIFIGAVTFTGSIIAYLKLSARMKGAPLTLPGRNLLNLAIIVLSVVGMVFFILTGTEEADNKAVAWTILGIMIVLALLLGLHLVAAIGGGDMPVVVSMLNSYSGWAAAAAGFMLANPLLIITGALVGLSGAYLSYIMCKAMNRSFISVILGGFGTEASSSDDRDYGTHTEITAEETAELLKGAKSVMITPGYGMAVAQAQYPVAAMVSKLREKGVDVTFGIHPVAGRLPGHMNVLLAEAKVPYDIVHEMDEVNDDFADIDVVLVIGANDTVNPIAEEPGSPLAGMPVLKVWEAKRVVVFKRSMGAGYAGVQNPLFFNENTDMLLGDAKDSVEKITSAL

SEQ ID NO: 97 - DNA, 1500 bp, synthetic construct
  source 1..1500: mol_type = other DNA
atgaactcttttattctggcgaccgaagtgaccaaccccgatgtgtctcaggatttgctggactggaccgaccgtatttctaccctcgcttaccttgtggcagccctgctcttcatcctcgctttggcgggtctgtctaagcagcaatccgctgcgcgcggcaacaccttcggtatcgctggtatgaccattgcgctcgttgcaaccgtgtttaaagcagccgtgcagtcccacgcagatccagagaactataatgacgcatgggtcaccatcttgcttgtcgcagttgccatgctgattggtgcagtcatcggcattgctcgcgcgtccaaggttgagatgaccggtatgccagaactcatcgccatgttgcactgcttcgtgggtgctgcggcagtgctgatcggcgtcaactcttttattcacgcggaacacacctccgaggcaggttacgaaaaattccaccttggcgaagtgtatctgggtatcttcattggcgcagtcacctttaccggctctatcattgcctaccttaagctgtccgcccgcatgaaaggtgctccgctcaccttgcccggccgtaacctgctcaatctcgcaatcattgtgttgtccgtggtcggtatggtcttctttatcctgaccggcaccgaagaggcagataacaaggcagttgcctggaccattcttggtatcatgattgtgctggccttgcttctgggtcttcacctggtcgcagctatcggtggtggtgacatgccggttgtggtctccatgctcaactcttactccggttgggcggcagccgctgcgggcttcatgttggctaatcccctcttgatcattaccggcgccctcgtcggtctttctggtgcttacttgtcctatatcatgtgtaaggctatgaaccgctctttcatctccgttattctgggtggctttggcaccgaagcgtcctcttccgatgaccgtgattatggcacccacaccgaggtcaccgcggaagagaccgcagaacttctgaagaacgccaaatccgttatgatcacccctggttacggtatggctgtggcacaggcacaatatcccgttgcagcaatggtgtccaagctgcgcgagaagggtgtggacgtcaccttcggcatccacccagtcgcaggtcgtctccctggccacatgaacgttctcttggccgaagctaaggtcccgtacgatattgttcacgaaatggacgaagtgaatgatgactttgccgacatcgacgttgtgctcgttattggcgccaacgataccgtgaatccaatcgctgaagagccaggttctcctattgcgggtatgccagtcttgaaggtttgggacgcaaaccgcgtcgttgtgttcaaacgctctatgggcgccggctacgctggcgttcaaaacccattgttctttaacgagaacaccgatatgcttctgggcgatgctaaggactctgtggaaaaaatcacctccgcgctgtaa

SEQ ID NO: 98 - protein, 499 aa, synthetic construct
MNSFILATEVTNPDVSQDLLDWTDRISTLAYLVAALLFILALAGLSKQQSASRGNTFGIAGMTIALVATVFKAAVQSHADPENYNDAWVTILLVAVAMLIGAVIGIARASKVEMTGMPELIAMLHCFVGAAAVLIGVNSFIHAEHTSEAGYEKFHLGEVYLGIFIGAVTFTGSIIAYLKLSARMKGAPLTLPGRNLLNLAIIVLSVVGMVFFILTGTEEADNKAVAWTILGIMIVLALLLGLHLVAAIGGGDMPVVVSMLNSYSGWAAAAAGFMLANPLLIITGALVGNSGAYLSYIMCKAMNRSFISVILGGFGTEASSSDDRDYGTHTEITAEETAELLKGAKSVMITPGYGMAVAQAQYPVAAMVSKLREKGVDVTFGIHPVAGRLPGHMNVLLAEAKVPYDIVHEMDEVNDDFADIDVVLVIGANDTVNPIAEEPGSPLAGMPVLKVWEAKRVVVFKRSMGAGYAGVQNPLFFNENTDMLLGDAKDSVEKITSAL

SEQ ID NO: 99 - DNA, 1500 bp, synthetic construct
  source 1..1500: mol_type = other DNA
atgaactcttttattctggcgaccgaagtgaccaaccccgatgtgtctcaggatttgctggactggaccgaccgtatttctaccctcgcttaccttgtggcagccctgctcttcatcctcgctttggcgggtctgtctaagcagcaatccgctgcgcgcggcaacaccttcggtatcgctggtatgaccattgcgctcgttgcaaccgtgtttaaagcagccgtgcagtcccacgcagatccagagaactataatgacgcatgggtcaccatcttgcttgtcgcagttgccatgctgattggtgcagtcatcggcattgctcgcgcgtccaaggttgagatgaccggtatgccagaactcatcgccatgttgcactgcttcgtgggtgctgcggcagtgctgatcggcgtcaactcttttattcacgcggaacacacctccgaggcaggttacgaaaaattccaccttggcgaagtgtatctgggtatcttcattggcgcagtcacctttaccggctctatcattgcctaccttaagctgtccgcccgcatgaaaggtgctccgctcaccttgcccggccgtaacctgctcaatctcgcaatcattgtgttgtccgtggtcggtatggtcttctttatcctgaccggcaccgaagaggcagataacaaggcagttgcctggaccattcttggtatcatgattgtgctggccttgcttctgggtcttcacctggtcgcagctatcggtggtggtgacatgccggttgtggtctccatgctcaactcttactccggttgggcggcagccgctgcgggcttcatgttggctaatcccctcttgatcattaccggcgccctcgtcggtaattctggtgcttacttgtcctatatcatgtgtaaggctatgaaccgctctttcatctccgttattctgggtggctttggcaccgaagcgtcctcttccgatgaccgtgattatggcacccacaccgaggtcaccgcggaagagaccgcagaacttctgaagaacgccaaatccgttatgatcacccctggttacggtatggctgtggcacaggcacaatatcccgttgcagcaatggtgtccaagctgcgcgagaagggtgtggacgtcaccttcggcatccacccagtcgcaggtcgtctccctggccacatgaacgttctcttggccgaagctaaggtcccgtacgatattgttcacgaaatggacgaagtgaatgatgactttgccgacatcgacgttgtgctcgttattggcgccaacgataccgtgaatccaatcgctgaagagccaggttctcctattgcgggtatgccagtcttgaaggtttgggacgcaaaccgcgtcgttgtgttcaaacgctctatgggcgccggctacgctggcgttcaaaacccattgttctttaacgagaacaccgatatgcttctgggcgatgctaaggactctgtggaaaaaatcacctccgcgctgtaa

SEQ ID NO: 100 - protein, 499 aa, synthetic construct
MNSFILATEVTNPDVSQDLLDWTDRISTLAYLVAALLFILALAGLSKQQSASRGNTFGIAGMTIALVATVFKAAVQSHADPENYNDAWVTILLVAVAMLIGAVIGIARASKVEMTGMPELIAMLHCFVGAAAVLIGVNSFIHAEHTSEAGYEKFHLGEVYLGIFIGAVTFTGSIIAYLKLSARMKGAPLTLPGRNLLNLAIIVLSVVGMVFFILTGTEEADNKAVAWTILGIMIVLALLLGLHLVAAIGGGDMPVVVSMLNSYSGWAAAAAGFMLANPLLIITGALVGPSGAYLSYIMCKAMNRSFISVILGGFGTEASSSDDRDYGTHTEITAEETAELLKGAKSVMITPGYGMAVAQAQYPVAAMVSKLREKGVDVTFGIHPVAGRLPGHMNVLLAEAKVPYDIVHEMDEVNDDFADIDVVLVIGANDTVNPIAEEPGSPLAGMPVLKVWEAKRVVVFKRSMGAGYAGVQNPLFFNENTDMLLGDAKDSVEKITSAL

SEQ ID NO: 101 - DNA, 1500 bp, synthetic construct
  source 1..1500: mol_type = other DNA
atgaactcttttattctggcgaccgaagtgaccaaccccgatgtgtctcaggatttgctggactggaccgaccgtatttctaccctcgcttaccttgtggcagccctgctcttcatcctcgctttggcgggtctgtctaagcagcaatccgctgcgcgcggcaacaccttcggtatcgctggtatgaccattgcgctcgttgcaaccgtgtttaaagcagccgtgcagtcccacgcagatccagagaactataatgacgcatgggtcaccatcttgcttgtcgcagttgccatgctgattggtgcagtcatcggcattgctcgcgcgtccaaggttgagatgaccggtatgccagaactcatcgccatgttgcactgcttcgtgggtgctgcggcagtgctgatcggcgtcaactcttttattcacgcggaacacacctccgaggcaggttacgaaaaattccaccttggcgaagtgtatctgggtatcttcattggcgcagtcacctttaccggctctatcattgcctaccttaagctgtccgcccgcatgaaaggtgctccgctcaccttgcccggccgtaacctgctcaatctcgcaatcattgtgttgtccgtggtcggtatggtcttctttatcctgaccggcaccgaagaggcagataacaaggcagttgcctggaccattcttggtatcatgattgtgctggccttgcttctgggtcttcacctggtcgcagctatcggtggtggtgacatgccggttgtggtctccatgctcaactcttactccggttgggcggcagccgctgcgggcttcatgttggctaatcccctcttgatcattaccggcgccctcgtcggtccctctggtgcttacttgtcctatatcatgtgtaaggctatgaaccgctctttcatctccgttattctgggtggctttggcaccgaagcgtcctcttccgatgaccgtgattatggcacccacaccgaggtcaccgcggaagagaccgcagaacttctgaagaacgccaaatccgttatgatcacccctggttacggtatggctgtggcacaggcacaatatcccgttgcagcaatggtgtccaagctgcgcgagaagggtgtggacgtcaccttcggcatccacccagtcgcaggtcgtctccctggccacatgaacgttctcttggccgaagctaaggtcccgtacgatattgttcacgaaatggacgaagtgaatgatgactttgccgacatcgacgttgtgctcgttattggcgccaacgataccgtgaatccaatcgctgaagagccaggttctcctattgcgggtatgccagtcttgaaggtttgggacgcaaaccgcgtcgttgtgttcaaacgctctatgggcgccggctacgctggcgttcaaaacccattgttctttaacgagaacaccgatatgcttctgggcgatgctaaggactctgtggaaaaaatcacctccgcgctgtaa

SEQ ID NO: 102 - protein, 499 aa, synthetic construct
MNSFILATEVTNPDVSQDLLDWTDRISTLAYLVAALLFILALAGLSKQQSASRGNTFGIAGMTIALVATVFKAAVQSHADPENYNDAWVTILLVAVAMLIGAVIGIARASKVEMTGMPELIAMLHCFVGAAAVLIGVNSFIHAEHTSEAGYEKFHLGEVYLGIFIGAVTFTGSIIAYLKLSARMKGAPLTLPGRNLLNLAIIVLSVVGMVFFILTGTEEADNKAVAWTILGIMIVLALLLGLHLVAAIGGGDMPVVVSMLNSYSGWAAAAAGFMLANPLLIITGALVGQSGAYLSYIMCKAMNRSFISVILGGFGTEASSSDDRDYGTHTEITAEETAELLKGAKSVMITPGYGMAVAQAQYPVAAMVSKLREKGVDVTFGIHPVAGRLPGHMNVLLAEAKVPYDIVHEMDEVNDDFADIDVVLVIGANDTVNPIAEEPGSPLAGMPVLKVWEAKRVVVFKRSMGAGYAGVQNPLFFNENTDMLLGDAKDSVEKITSAL

SEQ ID NO: 103 - DNA, 1500 bp, synthetic construct
  source 1..1500: mol_type = other DNA
atgaactcttttattctggcgaccgaagtgaccaaccccgatgtgtctcaggatttgctggactggaccgaccgtatttctaccctcgcttaccttgtggcagccctgctcttcatcctcgctttggcgggtctgtctaagcagcaatccgctgcgcgcggcaacaccttcggtatcgctggtatgaccattgcgctcgttgcaaccgtgtttaaagcagccgtgcagtcccacgcagatccagagaactataatgacgcatgggtcaccatcttgcttgtcgcagttgccatgctgattggtgcagtcatcggcattgctcgcgcgtccaaggttgagatgaccggtatgccagaactcatcgccatgttgcactgcttcgtgggtgctgcggcagtgctgatcggcgtcaactcttttattcacgcggaacacacctccgaggcaggttacgaaaaattccaccttggcgaagtgtatctgggtatcttcattggcgcagtcacctttaccggctctatcattgcctaccttaagctgtccgcccgcatgaaaggtgctccgctcaccttgcccggccgtaacctgctcaatctcgcaatcattgtgttgtccgtggtcggtatggtcttctttatcctgaccggcaccgaagaggcagataacaaggcagttgcctggaccattcttggtatcatgattgtgctggccttgcttctgggtcttcacctggtcgcagctatcggtggtggtgacatgccggttgtggtctccatgctcaactcttactccggttgggcggcagccgctgcgggcttcatgttggctaatcccctcttgatcattaccggcgccctcgtcggtcaatctggtgcttacttgtcctatatcatgtgtaaggctatgaaccgctctttcatctccgttattctgggtggctttggcaccgaagcgtcctcttccgatgaccgtgattatggcacccacaccgaggtcaccgcggaagagaccgcagaacttctgaagaacgccaaatccgttatgatcacccctggttacggtatggctgtggcacaggcacaatatcccgttgcagcaatggtgtccaagctgcgcgagaagggtgtggacgtcaccttcggcatccacccagtcgcaggtcgtctccctggccacatgaacgttctcttggccgaagctaaggtcccgtacgatattgttcacgaaatggacgaagtgaatgatgactttgccgacatcgacgttgtgctcgttattggcgccaacgataccgtgaatccaatcgctgaagagccaggttctcctattgcgggtatgccagtcttgaaggtttgggacgcaaaccgcgtcgttgtgttcaaacgctctatgggcgccggctacgctggcgttcaaaacccattgttctttaacgagaacaccgatatgcttctgggcgatgctaaggactctgtggaaaaaatcacctccgcgctgtaa

SEQ ID NO: 104 - protein, 499 aa, synthetic construct
MNSFILATEVTNPDVSQDLLDWTDRISTLAYLVAALLFILALAGLSKQQSASRGNTFGIAGMTIALVATVFKAAVQSHADPENYNDAWVTILLVAVAMLIGAVIGIARASKVEMTGMPELIAMLHCFVGAAAVLIGVNSFIHAEHTSEAGYEKFHLGEVYLGIFIGAVTFTGSIIAYLKLSARMKGAPLTLPGRNLLNLAIIVLSVVGMVFFILTGTEEADNKAVAWTILGIMIVLALLLGLHLVAAIGGGDMPVVVSMLNSYSGWAAAAAGFMLANPLLIITGALVGRSGAYLSYIMCKAMNRSFISVILGGFGTEASSSDDRDYGTHTEITAEETAELLKGAKSVMITPGYGMAVAQAQYPVAAMVSKLREKGVDVTFGIHPVAGRLPGHMNVLLAEAKVPYDIVHEMDEVNDDFADIDVVLVIGANDTVNPIAEEPGSPLAGMPVLKVWEAKRVVVFKRSMGAGYAGVQNPLFFNENTDMLLGDAKDSVEKITSAL

SEQ ID NO: 105 - DNA, 1500 bp, synthetic construct
  source 1..1500: mol_type = other DNA
atgaactcttttattctggcgaccgaagtgaccaaccccgatgtgtctcaggatttgctggactggaccgaccgtatttctaccctcgcttaccttgtggcagccctgctcttcatcctcgctttggcgggtctgtctaagcagcaatccgctgcgcgcggcaacaccttcggtatcgctggtatgaccattgcgctcgttgcaaccgtgtttaaagcagccgtgcagtcccacgcagatccagagaactataatgacgcatgggtcaccatcttgcttgtcgcagttgccatgctgattggtgcagtcatcggcattgctcgcgcgtccaaggttgagatgaccggtatgccagaactcatcgccatgttgcactgcttcgtgggtgctgcggcagtgctgatcggcgtcaactcttttattcacgcggaacacacctccgaggcaggttacgaaaaattccaccttggcgaagtgtatctgggtatcttcattggcgcagtcacctttaccggctctatcattgcctaccttaagctgtccgcccgcatgaaaggtgctccgctcaccttgcccggccgtaacctgctcaatctcgcaatcattgtgttgtccgtggtcggtatggtcttctttatcctgaccggcaccgaagaggcagataacaaggcagttgcctggaccattcttggtatcatgattgtgctggccttgcttctgggtcttcacctggtcgcagctatcggtggtggtgacatgccggttgtggtctccatgctcaactcttactccggttgggcggcagccgctgcgggcttcatgttggctaatcccctcttgatcattaccggcgccctcgtcggtcgttctggtgcttacttgtcctatatcatgtgtaaggctatgaaccgctctttcatctccgttattctgggtggctttggcaccgaagcgtcctcttccgatgaccgtgattatggcacccacaccgaggtcaccgcggaagagaccgcagaacttctgaagaacgccaaatccgttatgatcacccctggttacggtatggctgtggcacaggcacaatatcccgttgcagcaatggtgtccaagctgcgcgagaagggtgtggacgtcaccttcggcatccacccagtcgcaggtcgtctccctggccacatgaacgttctcttggccgaagctaaggtcccgtacgatattgttcacgaaatggacgaagtgaatgatgactttgccgacatcgacgttgtgctcgttattggcgccaacgataccgtgaatccaatcgctgaagagccaggttctcctattgcgggtatgccagtcttgaaggtttgggacgcaaaccgcgtcgttgtgttcaaacgctctatgggcgccggctacgctggcgttcaaaacccattgttctttaacgagaacaccgatatgcttctgggcgatgctaaggactctgtggaaaaaatcacctccgcgctgtaa

SEQ ID NO: 106 - protein, 499 aa, synthetic construct
MNSFILATEVTNPDVSQDLLDWTDRISTLAYLVAALLFILALAGLSKQQSASRGNTFGIAGMTIALVATVFKAAVQSHADPENYNDAWVTILLVAVAMLIGAVIGIARASKVEMTGMPELIAMLHCFVGAAAVLIGVNSFIHAEHTSEAGYEKFHLGEVYLGIFIGAVTFTGSIIAYLKLSARMKGAPLTLPGRNLLNLAIIVLSVVGMVFFILTGTEEADNKAVAWTILGIMIVLALLLGLHLVAAIGGGDMPVVVSMLNSYSGWAAAAAGFMLANPLLIITGALVGVSGAYLSYIMCKAMNRSFISVILGGFGTEASSSDDRDYGTHTEITAEETAELLKGAKSVMITPGYGMAVAQAQYPVAAMVSKLREKGVDVTFGIHPVAGRLPGHMNVLLAEAKVPYDIVHEMDEVNDDFADIDVVLVIGANDTVNPIAEEPGSPLAGMPVLKVWEAKRVVVFKRSMGAGYAGVQNPLFFNENTDMLLGDAKDSVEKITSAL

SEQ ID NO: 107 - DNA, 1500 bp, synthetic construct
  source 1..1500: mol_type = other DNA
atgaactcttttattctggcgaccgaagtgaccaaccccgatgtgtctcaggatttgctggactggaccgaccgtatttctaccctcgcttaccttgtggcagccctgctcttcatcctcgctttggcgggtctgtctaagcagcaatccgctgcgcgcggcaacaccttcggtatcgctggtatgaccattgcgctcgttgcaaccgtgtttaaagcagccgtgcagtcccacgcagatccagagaactataatgacgcatgggtcaccatcttgcttgtcgcagttgccatgctgattggtgcagtcatcggcattgctcgcgcgtccaaggttgagatgaccggtatgccagaactcatcgccatgttgcactgcttcgtgggtgctgcggcagtgctgatcggcgtcaactcttttattcacgcggaacacacctccgaggcaggttacgaaaaattccaccttggcgaagtgtatctgggtatcttcattggcgcagtcacctttaccggctctatcattgcctaccttaagctgtccgcccgcatgaaaggtgctccgctcaccttgcccggccgtaacctgctcaatctcgcaatcattgtgttgtccgtggtcggtatggtcttctttatcctgaccggcaccgaagaggcagataacaaggcagttgcctggaccattcttggtatcatgattgtgctggccttgcttctgggtcttcacctggtcgcagctatcggtggtggtgacatgccggttgtggtctccatgctcaactcttactccggttgggcggcagccgctgcgggcttcatgttggctaatcccctcttgatcattaccggcgccctcgtcggtgtgtctggtgcttacttgtcctatatcatgtgtaaggctatgaaccgctctttcatctccgttattctgggtggctttggcaccgaagcgtcctcttccgatgaccgtgattatggcacccacaccgaggtcaccgcggaagagaccgcagaacttctgaagaacgccaaatccgttatgatcacccctggttacggtatggctgtggcacaggcacaatatcccgttgcagcaatggtgtccaagctgcgcgagaagggtgtggacgtcaccttcggcatccacccagtcgcaggtcgtctccctggccacatgaacgttctcttggccgaagctaaggtcccgtacgatattgttcacgaaatggacgaagtgaatgatgactttgccgacatcgacgttgtgctcgttattggcgccaacgataccgtgaatccaatcgctgaagagccaggttctcctattgcgggtatgccagtcttgaaggtttgggacgcaaaccgcgtcgttgtgttcaaacgctctatgggcgccggctacgctggcgttcaaaacccattgttctttaacgagaacaccgatatgcttctgggcgatgctaaggactctgtggaaaaaatcacctccgcgctgtaa

SEQ ID NO: 108 - protein, 499 aa, synthetic construct
MNSFILATEVTNPDVSQDLLDWTDRISTLAYLVAALLFILALAGLSKQQSASRGNTFGIAGMTIALVATVFKAAVQSHADPENYNDAWVTILLVAVAMLIGAVIGIARASKVEMTGMPELIAMLHCFVGAAAVLIGVNSFIHAEHTSEAGYEKFHLGEVYLGIFIGAVTFTGSIIAYLKLSARMKGAPLTLPGRNLLNLAIIVLSVVGMVFFILTGTEEADNKAVAWTILGIMIVLALLLGLHLVAAIGGGDMPVVVSMLNSYSGWAAAAAGFMLANPLLIITGALVGWSGAYLSYIMCKAMNRSFISVILGGFGTEASSSDDRDYGTHTEITAEETAELLKGAKSVMITPGYGMAVAQAQYPVAAMVSKLREKGVDVTFGIHPVAGRLPGHMNVLLAEAKVPYDIVHEMDEVNDDFADIDVVLVIGANDTVNPIAEEPGSPLAGMPVLKVWEAKRVVVFKRSMGAGYAGVQNPLFFNENTDMLLGDAKDSVEKITSAL

SEQ ID NO: 109 - DNA, 1500 bp, synthetic construct
  source 1..1500: mol_type = other DNA
atgaactcttttattctggcgaccgaagtgaccaaccccgatgtgtctcaggatttgctggactggaccgaccgtatttctaccctcgcttaccttgtggcagccctgctcttcatcctcgctttggcgggtctgtctaagcagcaatccgctgcgcgcggcaacaccttcggtatcgctggtatgaccattgcgctcgttgcaaccgtgtttaaagcagccgtgcagtcccacgcagatccagagaactataatgacgcatgggtcaccatcttgcttgtcgcagttgccatgctgattggtgcagtcatcggcattgctcgcgcgtccaaggttgagatgaccggtatgccagaactcatcgccatgttgcactgcttcgtgggtgctgcggcagtgctgatcggcgtcaactcttttattcacgcggaacacacctccgaggcaggttacgaaaaattccaccttggcgaagtgtatctgggtatcttcattggcgcagtcacctttaccggctctatcattgcctaccttaagctgtccgcccgcatgaaaggtgctccgctcaccttgcccggccgtaacctgctcaatctcgcaatcattgtgttgtccgtggtcggtatggtcttctttatcctgaccggcaccgaagaggcagataacaaggcagttgcctggaccattcttggtatcatgattgtgctggccttgcttctgggtcttcacctggtcgcagctatcggtggtggtgacatgccggttgtggtctccatgctcaactcttactccggttgggcggcagccgctgcgggcttcatgttggctaatcccctcttgatcattaccggcgccctcgtcggttggtctggtgcttacttgtcctatatcatgtgtaaggctatgaaccgctctttcatctccgttattctgggtggctttggcaccgaagcgtcctcttccgatgaccgtgattatggcacccacaccgaggtcaccgcggaagagaccgcagaacttctgaagaacgccaaatccgttatgatcacccctggttacggtatggctgtggcacaggcacaatatcccgttgcagcaatggtgtccaagctgcgcgagaagggtgtggacgtcaccttcggcatccacccagtcgcaggtcgtctccctggccacatgaacgttctcttggccgaagctaaggtcccgtacgatattgttcacgaaatggacgaagtgaatgatgactttgccgacatcgacgttgtgctcgttattggcgccaacgataccgtgaatccaatcgctgaagagccaggttctcctattgcgggtatgccagtcttgaaggtttgggacgcaaaccgcgtcgttgtgttcaaacgctctatgggcgccggctacgctggcgttcaaaacccattgttctttaacgagaacaccgatatgcttctgggcgatgctaaggactctgtggaaaaaatcacctccgcgctgtaa

SEQ ID NO: 110 - protein, 499 aa, synthetic construct
MNSFILATEVTNPDVSQDLLDWTDRISTLAYLVAALLFILALAGLSKQQSASRGNTFGIAGMTIALVATVFKAAVQSHADPENYNDAWVTILLVAVAMLIGAVIGIARASKVEMTGMPELIAMLHCFVGAAAVLIGVNSFIHAEHTSEAGYEKFHLGEVYLGIFIGAVTFTGSIIAYLKLSARMKGAPLTLPGRNLLNLAIIVLSVVGMVFFILTGTEEADNKAVAWTILGIMIVLALLLGLHLVAAIGGGDMPVVVSMLNSYSGWAAAAAGFMLANPLLIITGALVGYSGAYLSYIMCKAMNRSFISVILGGFGTEASSSDDRDYGTHTEITAEETAELLKGAKSVMITPGYGMAVAQAQYPVAAMVSKLREKGVDVTFGIHPVAGRLPGHMNVLLAEAKVPYDIVHEMDEVNDDFADIDVVLVIGANDTVNPIAEEPGSPLAGMPVLKVWEAKRVVVFKRSMGAGYAGVQNPLFFNENTDMLLGDAKDSVEKITSAL

SEQ ID NO: 111 - DNA, 1500 bp, synthetic construct
  source 1..1500: mol_type = other DNA
atgaactcttttattctggcgaccgaagtgaccaaccccgatgtgtctcaggatttgctggactggaccgaccgtatttctaccctcgcttaccttgtggcagccctgctcttcatcctcgctttggcgggtctgtctaagcagcaatccgctgcgcgcggcaacaccttcggtatcgctggtatgaccattgcgctcgttgcaaccgtgtttaaagcagccgtgcagtcccacgcagatccagagaactataatgacgcatgggtcaccatcttgcttgtcgcagttgccatgctgattggtgcagtcatcggcattgctcgcgcgtccaaggttgagatgaccggtatgccagaactcatcgccatgttgcactgcttcgtgggtgctgcggcagtgctgatcggcgtcaactcttttattcacgcggaacacacctccgaggcaggttacgaaaaattccaccttggcgaagtgtatctgggtatcttcattggcgcagtcacctttaccggctctatcattgcctaccttaagctgtccgcccgcatgaaaggtgctccgctcaccttgcccggccgtaacctgctcaatctcgcaatcattgtgttgtccgtggtcggtatggtcttctttatcctgaccggcaccgaagaggcagataacaaggcagttgcctggaccattcttggtatcatgattgtgctggccttgcttctgggtcttcacctggtcgcagctatcggtggtggtgacatgccggttgtggtctccatgctcaactcttactccggttgggcggcagccgctgcgggcttcatgttggctaatcccctcttgatcattaccggcgccctcgtcggttactctggtgcttacttgtcctatatcatgtgtaaggctatgaaccgctctttcatctccgttattctgggtggctttggcaccgaagcgtcctcttccgatgaccgtgattatggcacccacaccgaggtcaccgcggaagagaccgcagaacttctgaagaacgccaaatccgttatgatcacccctggttacggtatggctgtggcacaggcacaatatcccgttgcagcaatggtgtccaagctgcgcgagaagggtgtggacgtcaccttcggcatccacccagtcgcaggtcgtctccctggccacatgaacgttctcttggccgaagctaaggtcccgtacgatattgttcacgaaatggacgaagtgaatgatgactttgccgacatcgacgttgtgctcgttattggcgccaacgataccgtgaatccaatcgctgaagagccaggttctcctattgcgggtatgccagtcttgaaggtttgggacgcaaaccgcgtcgttgtgttcaaacgctctatgggcgccggctacgctggcgttcaaaacccattgttctttaacgagaacaccgatatgcttctgggcgatgctaaggactctgtggaaaaaatcacctccgcgctgtaa

SEQ ID NO: 112 - DNA, 5802 bp, synthetic construct
  source 1..5802: mol_type = other DNA
gttcgcttgctgtccataaaaccgcccagtctagctatcgccatgtaagcccactgcaagctacctgctttctctttgcgcttgcgttttcccttgtccagatagcccagtagctgacattcatccggggtcagcaccgtttctgcggactggctttctacgtgttccgcttcctttagcagcccttgcgccctgagtgcttgcggcagcgtgaagctagcttttatcgccattcgccattcaggctgcgcaactgttgggaagggcgatcggtgcgggcctcttcgctattacgccagctggcgaaagggggatgtgctgcaaggcgattaagttgggtaacgccagggttttcccagtcacgacgttgtaaaacgacggccagtgaattcgagctcggtacccggggatcctctagagtcgacctgcaggcatgcaagcttggcgtaatcatggtcatagctgtttcctgtgtgaaattgttatccgctcacaattccacacaacatacgagccggaagcataaagtgtaaagcctggggtgcctaatgagtgagctaactcacattaattgcgttgcgctcactgcccgctttccagtcgggaaacctgtcgtgccagctgcattaatgaatcggccaacgcgcggggagaggcggtttgcgtattgggcgctcttccgcttcctcgctcactgactcgctgcgctcggtcgttcggctgcggcgagcggtatcagctcactcaaaggcggtaatacggttatccacagaatcaggggataacgcaggaaagaacatgtgagcaaaaggccagcaaaaggccaggaaccgtaaaaaggccgcgttgctggcgtttttccataggctccgcccccctgacgagcatcacaaaaatcgacgctcaagtcagaggtggcgaaacccgacaggactataaagataccaggcgtttccccctggaagctccctcgtgcgctctcctgttccgaccctgccgcttaccggatacctgtccgcctttctcccttcgggaagcgtggcgctttctcaatgctcacgctgtaggtatctcagttcggtgtaggtcgttcgctccaagctgggctgtgtgcacgaaccccccgttcagcccgaccgctgcgccttatccggtaactatcgtcttgagtccaacccggtaagacacgacttatcgccactggcagcagccactggtaacaggattagcagagcgaggtatgtaggcggtgctacagagttcttgaagtggtggcctaactacggctacactagaaggacagtatttggtatctgcgctctgctgaagccagttaccttcggaaaaagagttggtagctcttgatccggcaaacaaaccaccgctggtagcggtggtttttttgtttgcaagcagcagattacgcgcagaaaaaaaggatctcaagaagatcctttgatcttttctacggggtctgacgctcagtggaacgaaaactcacgttaagggattttggtcatgagattatcaaaaaggatcttcacctagatccttttggggtgggcgaagaactccagcatgagatccccgcgctggaggatcatccagccctgatagaaacagaagccactggagcacctcaaaaacaccatcatacactaaatcagtaagttggcagcatcacccgacgcactttgcgccgaataaatacctgtgacggaagatcacttcgcagaataaataaatcctggtgtccctgttgataccgggaagccctgggccaacttttggcgaaaatgagacgttgatcggcacgtaagaggttccaactttcaccataatgaaataagatcactaccgggcgtattttttgagttatcgagattttcaggagctgatagaaacagaagccactggagcacctcaaaaacaccatcatacactaaatcagtaagttggcagcatcacccgacgcactttgcgccgaataaatacctgtgacggaagatcacttcgcagaataaataaatcctggtgtccctgttgataccgggaagccctgggccaacttttggcgaaaatgagacgttgatcggcacgtaagaggttccaactttcaccataatgaaataagatcactaccgggcgtattttttgagttatcgagattttcaggagctctttggcatcgtctctcgcctgtcccctcagttcagtaatttcctgcatttgcctgtttccagtcggtagatattccacaaaacagcagggaagcagcgcttttccgctgcataaccctgcttcggggtcattatagcgattttttcggtatatccatcctttttcgcacgatatacaggattttgccaaagggttcgtgtagactttccttggtgtatccaacggcgtcagccgggcaggataggtgaagtaggcccacccgcgagcgggtgttccttcttcactgtcccttattcgcacctggcggtgctcaacgggaatcctgctctgcgaggctggccggctaccgccggcgtaacagatgagggcaagcggatggctgatgaaaccaagccaaccaggaagggcagcccacctatcaaggtgtactgccttccagacgaacgaagagcgattgaggaaaaggcggcggcggccggcatgagcctgtcggcctacctgctggccgtcggccagggctacaaaatcacgggcgtcgtggactatgagcacgtccgcgagggcgtcccggaaaacgattccgaagcccaacctttcatagaaggcggcggtggaatcgaaatctcgtgatggcaggttgggcgtcgcttggtcggtcatttcgaaaaaggttaggaatacggttagccatttgcctgcttttatatagttcatatgggattcacctttatgttgataagaaataaaagaaaatgccaataggatatcggcattttcttttgcgtttttatttgttaactgttaattgtccttgttcaaggatgctgtctttgacaacagatgttttcttgcctttgatgttcagcaggaagctcggcgcaaacgttgattgtttgtctgcgtagaatcctctgtttgtcatatagcttgtaatcacgacattgtttcctttcgcttgaggtacagcgaagtgtgagtaagtaaaggttacatcgttaggcggatcaagatccatttttaacacaaggccagttttgttcagcggcttgtatgggccagttaaagaattagaaacataaccaagcatgtaaatatcgttagacgtaatgccgtcaatcgtcatttttgatccgcgggagtcagtgaacaggtaccatttgccgttcattttaaagacgttcgcgcgttcaatttcatctgttactgtgttagatgcaatcagcggtttcatcacttttttcagtgtgtaatcatcgtttagctcaatcataccgagagcgccgtttgctaactcagccgtgcgttttttatcgctttgcagaagtttttgactttcttgacggaagaatgatgtgcttttgccatagtatgctttgttaaataaagattcttcgccttggtagccatcttcagttccagtgtttgcttcaaatactaagtatttgtggcctttatcttctacgtagtgaggatctctcagcgtatggttgtcgcctgagctgtagttgccttcatcgatgaactgctgtacattttgatacgtttttccgtcaccgtcaaagattgatttataatcctctacaccgttgatgttcaaagagctgtctgatgctgatacgttaacttgtgcagttgtcagtgtttgtttgccgtaatgtttaccggagaaatcagtgtagaataaacggatttttccgtcagatgtaaatgtggctgaacctgaccattcttgtgtttggtcttttaggatagaatcatttgcatcgaatttgtcgctgtctttaaagacgcggccagcgtttttccagctgtcaatagaagtttcgccgactttttgatagaacatgtaaatcgatgtgtcatccgcatttttaggatctccggctaatgcaaagacgatgtggtagccgtgatagtttgcgacagtgccgtcagcgttttgtaatggccagctgtcccaaacgtccaggccttttgcagaagagatatttttaattgtggacgaatcaaattcagaaacttgatatttttcatttttttgctgttcagggatttgcagcatatcatggcgtgtaatatgggaaatgccgtatgtttccttatatggcttttggttcgtttctttcgcaaacgcttgagttgcgcctcctgccagcagtgcggtagtaaaggttaatactgttgcttgttttgcaaactttttgatgttcatcgttcatgtctccttttttatgtactgtgttagcggtctgcttcttccagccctcctgtttgaagatggcaagttagttacgcacaataaaaaaagacctaaaatatgtaaggggtgacgccaaagtatacactttgccctttacacattttaggtcttgcctgctttatcagtaacaaacccgcgcgatttacttttcgacctcattctattagactctcgtttggattgcaactggtctattttcctcttttgtttgatagaaaatcataaaaggatttgcagactacgggcctaaagaactaaaaaatctatctgtttcttttcattctctgtattttttatagtttctgttgcatgggcataaagttgcctttttaatcacaattcagaaaatatcataatatctcatttcactaaataatagtgaacggcaggtatatgtgatgggttaaaaaggatcaccccagagtcccgctcagaagaactcgtcaagaaggcgatagaaggcgatgcgctgcgaatcgggagcggcgataccgtaaagcacgaggaagcggtcagcccattcgccgccaagctcttcagcaatatcacgggtagccaacgctatgtcctgatagcggtccgccacacccagccggccacagtcgatgaatccagaaaagcggccattttccaccatgatattcggcaagcaggcatcgccatgggtcacgacgagatcctcgccgtcgggcatccgcgccttgagcctggcgaacagttcggctggcgcgagcccctgatgctcttcgtccagatcatcctgatcgacaagaccggcttccatccgagtacgtgctcgctcgatgcgatgtttcgcttggtggtcgaatgggcaggtagccggatcaagcgtatgcagccgccgcattgcatcagccatgatggatactttctcggcaggagcaaggtgagatgacaggagatcctgccccggcacttcgcccaatagcagccagtcccttcccgcttcagtgacaacgtcgagacagctgcgcaaggaacgcccgtcgtggccagccacgatagccgcgctgcctcgtcttggagttcattcagggcaccggacaggtcggtcttgacaaaaagaaccgggcgcccctgcgctgacagccggaacacggcggcatcagagcagccgattgtctgttgtgcccagtcatagccgaatagcctctccacccaagcggccggagaacctgcgtgcaatccatcttgttcaatcatgcgaaacgatcctcatcctgtctcttgatcagatcttgatcccctgcgccatcagatccttggcggcaagaaagccatccagtttactttgcagggcttcccaaccttaccagagggcgccccagctggcaattccg